European Patent Specification EP 3 756 665 B1, published August 14, 2024. Title: INTERVAL THERAPY FOR THE TREATMENT OF EYE DISEASES. Applicant: Ramot at Tel-Aviv University Ltd. The sequence listing filed with the application follows.

SEQUENCE LISTING (33 sequences)

SEQ ID NO: 1 - protein, 3 aa, Artificial Sequence
  Synthetic Peptide
  misc_feature (1)..(3): Stereoisomer D
FFP

SEQ ID NO: 2 - protein, 4 aa, Artificial Sequence
  Synthetic Peptide
  misc_feature (1)..(1): Alpha-aminoisobutyric acid (Aib)
  misc_feature (2)..(3): Stereoisomer D
  misc_feature (4)..(4): Alpha-aminoisobutyric acid (Aib)
XFNX

SEQ ID NO: 3 - protein, 3 aa, Artificial Sequence
  Synthetic Peptide
  misc_feature (1)..(3): Stereoisomer D
FNP

SEQ ID NO: 4 - protein, 4 aa, Artificial Sequence
  Synthetic Peptide
  misc_feature (1)..(1): Alpha-aminoisobutyric acid (Aib)
  misc_feature (4)..(4): Alpha-aminoisobutyric acid (Aib)
XNFX

SEQ ID NO: 5 - protein, 6 aa, Artificial Sequence
  Synthetic Peptide
QKLVFF

SEQ ID NO: 6 - protein, 2 aa, Artificial Sequence
  Synthetic Peptide
YY

SEQ ID NO: 7 - protein, 3 aa, Artificial Sequence
  Synthetic peptide
  misc_feature (1)..(3): Stereoisomer D
FFP

SEQ ID NO: 8 - protein, 4 aa, Artificial Sequence
  Synthetic Peptide
  misc_feature (1)..(1): Alpha-aminoisobutyric acid (Aib)
  misc_feature (2)..(3): Stereoisomer D
  misc_feature (4)..(4): Alpha-aminoisobutyric acid (Aib)
XFNX

SEQ ID NO: 9 - protein, 4 aa, Artificial Sequence
  Synthetic Peptide
  misc_feature (1)..(1): Alpha-aminoisobutyric acid (Aib)
  misc_feature (4)..(4): Alpha-aminoisobutyric acid (Aib)
XNFX

SEQ ID NO: 10 - protein, 2 aa, Artificial Sequence
  Synthetic Peptide
YY

SEQ ID NO: 11 - protein, 2 aa, Artificial Sequence
  Synthetic Peptide
  misc_feature (2)..(2): amidated amino acid
YY

SEQ ID NO: 12 - protein, 3 aa, Artificial Sequence
  Synthetic Peptide
  misc_feature (1)..(1): Alpha-aminoisobutyric acid (Aib)
XFF

SEQ ID NO: 13 - protein, 3 aa, Artificial Sequence
  Synthetic Peptide
  misc_feature (3)..(3): Alpha-aminoisobutyric acid (Aib)
NYX

SEQ ID NO: 14 - protein, 3 aa, Artificial Sequence
  Synthetic Peptide
NYP

SEQ ID NO: 15 - protein, 4 aa, Artificial Sequence
  Synthetic Peptide
  misc_feature (1)..(1): Beta-aminoisobutyric acid
  misc_feature (2)..(4): Stereoisomer D
XPYN

SEQ ID NO: 16 - protein, 2 aa, Artificial Sequence
  Synthetic Peptide
  misc_feature (1)..(1): Stereoisomer D
  misc_feature (2)..(2): Alpha-aminoisobutyric acid (Aib)
YX

SEQ ID NO: 17 - protein, 2 aa, Artificial Sequence
  Synthetic Peptide
  misc_feature (1)..(2): Stereoisomer D
PY

SEQ ID NO: 18 - protein, 2 aa, Artificial Sequence
  Synthetic Peptide
  misc_feature (1)..(2): Stereoisomer D
YP

SEQ ID NO: 19 - protein, 4 aa, Artificial Sequence
  Synthetic Peptide
NYYP

SEQ ID NO: 20 - protein, 3 aa, Artificial Sequence
  Synthetic Peptide
  misc_feature (3)..(3): Alpha-aminoisobutyric acid (Aib)
YYX

SEQ ID NO: 21 - protein, 3 aa, Artificial Sequence
  Synthetic Peptide
  misc_feature (1)..(1): Alpha-aminoisobutyric acid (Aib)
XYY

SEQ ID NO: 22 - protein, 4 aa, Artificial Sequence
  Synthetic Peptide
  misc_feature (1)..(1): Alpha-aminoisobutyric acid (Aib)
  misc_feature (4)..(4): Alpha-aminoisobutyric acid (Aib)
XYYX

SEQ ID NO: 23 - protein, 4 aa, Artificial Sequence
  Synthetic Peptide
  misc_feature (1)..(1): Stereoisomer D
  misc_feature (4)..(4): Stereoisomer D
NYYP

SEQ ID NO: 24 - protein, 3 aa, Artificial Sequence
  Synthetic Peptide
PYY

SEQ ID NO: 25 - protein, 3 aa, Artificial Sequence
  Synthetic Peptide
YYP

SEQ ID NO: 26 - protein, 4 aa, Artificial Sequence
  Synthetic Peptide
PYYP

SEQ ID NO: 27 - protein, 2 aa, Artificial Sequence
  Synthetic Peptide
  misc_feature (1)..(2): Stereoisomer D
YY

SEQ ID NO: 28 - protein, 2 aa, Artificial Sequence
  Synthetic Peptide
  misc_feature (1)..(1): Stereoisomer D
  misc_feature (2)..(2): Alpha-aminoisobutyric acid (Aib)
PX

SEQ ID NO: 29 - protein, 2 aa, Artificial Sequence
  Synthetic Peptide
  misc_feature (1)..(2): Stereoisomer D
FP

SEQ ID NO: 30 - protein, 2 aa, Artificial Sequence
  Synthetic Peptide
  misc_feature (1)..(1): Stereoisomer D
  misc_feature (2)..(2): Alpha-aminoisobutyric acid (Aib)
WX

SEQ ID NO: 31 - protein, 2 aa, Artificial Sequence
  Synthetic Peptide
  misc_feature (1)..(2): Stereoisomer D
WP

SEQ ID NO: 32 - protein, 2 aa, Artificial Sequence
  Synthetic Peptide
  misc_feature (1)..(1): Stereoisomer D
FP

SEQ ID NO: 33 - protein, 2 aa, Artificial Sequence
  Synthetic Peptide
  misc_feature (2)..(2): Stereoisomer D
PF